European Patent Application EP 4 130 264 A1, published February 8, 2023. Title: Novel adrenomedullin analogues, a method for the production thereof and a medical use thereof. Applicant: University of Miyazaki. The sequence listing filed with the application follows.

SEQUENCE LISTING (11 sequences)

SEQ ID NO: 1 - protein, 52 aa, Homo sapiens
YRQSMNNFQGLRSFGCRFGTCTVQKLAHQIYQFTDKDKDNVAPRSKISPQGY

SEQ ID NO: 2 - protein, 32 aa, Artificial
  Synthetic
SFGCRFGTCTVQKLAHQIYQFTDKDKDNVAPR

SEQ ID NO: 3 - protein, 40 aa, Artificial
  Synthetic
SFGCRFGTCTVQKLAHQIYQFTDKDKDNVAPRSKISPQGY

SEQ ID NO: 4 - protein, 40 aa, Artificial
  Synthetic
  misc_feature (32)..(32): Xaa is D-Arg
SFGCRFGTCTVQKLAHQIYQFTDKDKDNVAPXSKISPQGY

SEQ ID NO: 5 - protein, 40 aa, Artificial
  Synthetic
SFGCRFGTCTVQKLAHQIYQFTDKDKDNVAPKSKISPQGY

SEQ ID NO: 6 - protein, 40 aa, Artificial
  Synthetic
SFGCRFGTCTVQKLAHQIYQFTDKDKDNVAPASKISPQGY

SEQ ID NO: 7 - protein, 40 aa, Artificial
  Synthetic
SFGCRFGTCTVQKLAHQIYQFTDKDKDNVAPGSKISPQGY

SEQ ID NO: 8 - protein, 39 aa, Artificial
  Synthetic
SFGCRFGTCTVQKLAHQIYQFTDKDKDNVAPSKISPQGY

SEQ ID NO: 9 - protein, 40 aa, Artificial
  Synthetic
SFGCRFGTCTVQKLAHQIYQFTDKDKDNVAPDSKISPQGY

SEQ ID NO: 10 - protein, 40 aa, Artificial
  Synthetic
SFGCRFGTCTVQKLAHQIYQFTDKDKDNVAPFSKISPQGY

SEQ ID NO: 11 - protein, 40 aa, Artificial
  Synthetic
SFGCRFGTCTVQKLAHQIYQFTDKDKDNVAPRPKISPQGY